European Patent Specification EP 3 817 757 B1, published January 7, 2026. Title: PEPTIDE DEFICIENT-MHC CLASS I/CHAPERONE COMPOSITIONS AND METHODS. Applicant: The Regents of the University of California Sgourakis, Nikolaos G. Application PCT/US19/40616. The sequence listing filed with the application follows.

SEQUENCE LISTING (16 sequences)

SEQ ID NO: 1 - protein, 9 aa, Artificial Sequence
  gP18-I10 placeholder peptide
GPGRAFVTI

SEQ ID NO: 2 - protein, 9 aa, Artificial Sequence
  QL9 placeholder peptide
QLSPFPFDL

SEQ ID NO: 3 - protein, 8 aa, Artificial Sequence
  gTAX placeholder peptide
LFGYPVYV

SEQ ID NO: 4 - protein, 8 aa, Artificial Sequence
  acetylated TAX placeholder peptide
  MOD_RES (1)..(1): Leu is acetylated leucine
LFGYPVYV

SEQ ID NO: 5 - protein, 10 aa, Artificial Sequence
  HIV gp160 epitope P18-I10
RGPGRAFVTI

SEQ ID NO: 6 - protein, 8 aa, Artificial Sequence
  gp29
PNVNIHNF

SEQ ID NO: 7 - protein, 9 aa, Artificial Sequence
  TAX placeholder peptide
LLFGYPVYV

SEQ ID NO: 8 - protein, 8 aa, Artificial Sequence
  D-leucine synthetic TAX placeholder peptide
  MOD_RES (1)..(1): Leu is a D-leucine
LFGYPVYV

SEQ ID NO: 9 - protein, 9 aa, Artificial Sequence
  Synthetic peptide
  MOD_RES (8)..(8): Xaa is 3-amino-3-(2-nitrophenyl)-propionic acid
GILGFVFXL

SEQ ID NO: 10 - protein, 10 aa, Artificial Sequence
  photo-P18-I10
  MOD_RES (8)..(8): Xaa is 3-amino-3-(2-nitrophenyl)-propionic acid
RGPGRAFXTI

SEQ ID NO: 11 - DNA, 20 bp, Artificial Sequence
  tetramer additive
gtctcgtgggctcggagatg

SEQ ID NO: 12 - DNA, 19 bp, Artificial Sequence
  PCR - DMF5_PCR1 primer
gaaattcacggcgcacagg

SEQ ID NO: 13 - DNA, 43 bp, Artificial Sequence
  PCR2 -  DMF5_PCR2 primer
ccttggcacccgagaattccagcttggctggctgtctctgatc

SEQ ID NO: 14 - DNA, 29 bp, Artificial Sequence
  P5_generic primer
aatgatacggcgaccaccgagatctacac

SEQ ID NO: 15 - DNA, 64 bp, Artificial Sequence
  RPI-x primer
  misc_feature (25)..(31): n is a, c, g, or t
caagcagaagacggcatacgagatnnnnnnngtgactggagttccttggcacccgagaattcca

SEQ ID NO: 16 - DNA, 47 bp, Artificial Sequence
  N7XX primer
  misc_feature (25)..(32): n is a, c, g, or t
caagcagaagacggcatacgagatnnnnnnnngtctcgtgggctcgg